European Patent Application EP 4 717 774 A1, published April 1, 2026. Title: Method for producing PF1378A. Applicant: Mitsui Chemicals Crop & Life Solutions Inc. The sequence listing filed with the application follows.

SEQUENCE LISTING (9 sequences)

SEQ ID NO: 1 - DNA, 1554 bp, Aspergillus aculeatinus PF1378
  source 1..1554: mol_type = other DNA
atgctggaaaccttttgttccgggctggcatccatctcaacagccaacctcgcctcctcagcggtaatatgtacagcgctgtacctcgccggtgtggccgtttaccgtctctacctttcaccgatatcgcacttcccgggcccgaggctggccgcgttgacatgggcctacgagttctactacgactgggttctccccgggaagtactacgagcgagtagccgagatgcacaggcaatatgggtcaatcgtgcgagtcaccccggatgaactccatatcctcgacccctcatattacgacggggtttatgtaactgcagccacacggcggacggatgttccctatgactttggacttggcacaggattccacgatattgcacgaaatgctcagagccacgacgaccatcgtgggaactatcgattcctgaaagccttcttctcgcgagcttccatcacgcggctcgaaggcctgacgacggagcggttggatcggcttgatgcgcggttgcgagaatgggtggatgccgcggagccggtgaacctcacctatgcgatgtactcgtatgtgactgacatcatatcttcgatgctctttgaagagccatgcgacttcctgagtgacccggggttcaatgggtcctggttcgaaaagctgaaacacgggatggtcaatgttcctctgtttgcgttcatgccttggcttccaagaatcatcgccctgccactggtgagctacttgttcgacagagaaaagaggtgggctgtttttgatgaacgcacacaacgccagcaaatgactcgccgagatcggccgagcgacgcgacctcaactcgctcggggaagaccctgttcgacgagcttgtccgacagaaccagaccaaggtcccgttcgacgcggacgtttgtagggaggtggcccagtccttccagcaagccgccggccataatctgaaccgcaccctcgaggctaccattaccctgctcgccatggacaaagagcggcaagagaagttacgcacctcgctggagccagtctttgcgaatgcgcagcgcccatcctgggtggagcttgagaagatcccgtacctcacggcttgcgtacaggaggggattagactgggaggcggcaatctccgccgggcggcccgaatctcgccggatgaagatctggtctacaaggggtggaggattcccaaaaagactccggttgggatgacgatctactggatgctcatggatccggctgtgttcccgtcgccgagaacgtttaaccctgaacgctggctggaatgctccgatgaacaccttgcggagatgcactgccacttcgttgcgttcaccaagggatccaggagctgtattggtaaccacttaacgtacatggtcatgtatcacacgatcgcctggttgttccggcccggggcaccgcggatccagttgtacgagacagacgagagccacgtcctgtcgagttacggattattttttagtttgcccagggttgatataccgggggtgagggcatacttgacaaacaagtatgaggggtaa

SEQ ID NO: 2 - protein, 517 aa, Aspergillus aculeatinus PF1378
MLETFCSGLASISTANLASSAVICTALYLAGVAVYRLYLSPISHFPGPRLAALTWAYEFYYDWVLPGKYYERVAEMHRQYGSIVRVTPDELHILDPSYYDGVYVTAATRRTDVPYDFGLGTGFHDIARNAQSHDDHRGNYRFLKAFFSRASITRLEGLTTERLDRLDARLREWVDAAEPVNLTYAMYSYVTDIISSMLFEEPCDFLSDPGFNGSWFEKLKHGMVNVPLFAFMPWLPRIIALPLVSYLFDREKRWAVFDERTQRQQMTRRDRPSDATSTRSGKTLFDELVRQNQTKVPFDADVCREVAQSFQQAAGHNLNRTLEATITLLAMDKERQEKLRTSLEPVFANAQRPSWVELEKIPYLTACVQEGIRLGGGNLRRAARISPDEDLVYKGWRIPKKTPVGMTIYWMLMDPAVFPSPRTFNPERWLECSDEHLAEMHCHFVAFTKGSRSCIGNHLTYMVMYHTIAWLFRPGAPRIQLYETDESHVLSSYGLFFSLPRVDIPGVRAYLTNKYEG

SEQ ID NO: 3 - DNA, 2132 bp, Aspergillus aculeatinus PF1378
  source 1..2132: mol_type = genomic DNA
atgctggaaaccttttgttccgggctggcatccatctcaacagccaacctcgcctcctcagcggtaatatgtacagcgctgtacctcgccggtgtggccgtttaccgtctctacctttcaccgatatcgcacttcccgggcccgaggctggccgcgttgacatgggcctacgagttctactacgactgggttctccccgggaagtactacgagcgagtagccgagatgcacaggcaatatggtagctctcctgacattgactcggtaccagcaatcggactaacgagacctccagggtcaatcgtgcgagtcaccccggatgaactccatatcctcgacccctcatattacgacggggtttatgtaactgcagccacacggcggacggatgttccctatgactttggacttggcacaggattccacggtatccttgccgccgctccgtgttgtgtgctttccggtcactgactgcttcagatattgcacgaaatgctcagagccacgacgaccatcgtgggaactatcgattcctgaaagccttcttctcgcgagcttccatcacgcggctcgaaggcctgacgacggagcggttggatcggcttgatgcgcggttgcgagaatgggtggatgccgcggagccggtgaacctcacctatgcgatgtactcgtatgtgactggtgagtctgtgggatgtttcggcccactgatgcagatctaatctcccccggcgcagacatcatatcttcgatgctctttgaagagccatgcgacttcctgagtgacccggggttcaatgggtcctggttcgaaaagctgaaacacgggatggtcaatgttcctctgtttgcgttcatgccttggcttccaaggtttgtcaccccctccagctggttttctgcctatgtgtaaccgcgaggtagaatcatcgccctgccactggtgagctacttgttcgacagagaaaagaggtgggctgtttttgatgaagtatgcatccctcaccttattgcagcttgatatatgccccaaccgctgacgtctggcccggtcatcagcgcacacaacgccagcaaatgactcgccgagatcggccgagcgacgcgacctcaactcgctcggggaagaccctgttcgacgagcttgtccgacagaaccagaccaaggtcccgttcgacgcggacgtttgtagggaggtggcccaggtgcgtttggatggatctccattcaatcaaaaaataagaaagaatgaaagaaagaaaacatcataaaaaggttcaatcctgacgatttaaatcctttgcagtccttccagcaagccgccggccataatctgaaccgcaccctcgaggctaccattaccctgctcgccatggacaaagagcggcaagagaagttacgcacctcgctggagccagtctttgcgaatgcgcagcgcccatcctgggtggagcttgagaagatcccgtacctcacggcttgcgtacaggaggggattaggtcagtccaaactactaattgacatatatccaatcccgatctaattgatattggtagactgggaggcggcaatctccgccgggcggcccgaatctcgccggatgaagatctggtctacaaggggtggaggattcccaaaaaggtgtgtcgaggagagtctcactatgcaataccccggtctaatcacaaggcctccttccgctcctcagactccggttgggatgacgatctactggatgctcatggatccggctgtgttcccgtcgccgagaacgtttaaccctgaacgctggctggaatgctccgatgaacaccttgcggagatgcactgccacttcgttgcgttcaccaagggatccaggagctgtattggtaaccagtatgtataattccctttcccaccccagcgatgtcttgtgtgaccagaaggaagctgaaaaccggcgacagcttaacgtacatggtcatgtatcacacgatcgcctggttgttccggcccggggcaccgcggatccagttgtacgagacagacgagagccacgtcctgtcgagttacggattattttttagtttgcccagggttgatataccgggggtgagggcatacttgacaaacaagtatgaggggtaa

SEQ ID NO: 4 - DNA, 2245 bp, Aspergillus aculeatinus PF1378
  source 1..2245: mol_type = genomic DNA
atggccgacagtaacccaccgcgagacgatgaagtaggcgaagaggaagaagaggagatcgatgaatccgtacatacttccctttcgctcgattttttccaaatgaaaagcacagctaggctgatcccctatagaactacaaatcggtgaaagatgcggttctctttgcgatcgaagttagcgactccatgctcgagcctcgcccatctgccgaccccaagaaacccgtggaagaatcgccggtcaccgcagccttgaaatgcgcataccacttgatgcaacagcgaatcatttctaacccacaagatatgatgggagttctcttgtacgggacgcaggcgtccaagttctacgatgaagacgagggcagccgaggcgacttgtcctatcccaactgctacctcttcacagacctcgacatcccgtctgcgcaagaggtcaaggaccttcgagcgctggtagaagacgaggggaaaggcagagagattctcgtgccggcagagaagcaagtgtccatggcaaacgtcctattctgtgccaaccagattttcacctccaaagcgcccaacttcctttcgcggcggttgttcatagtcaccgacaacgacagtcctcacacccaagacaaagccctgcggtctgccgcgacagtgcgagctaaggatctatacgatctcggagtcactattgagctcttccctatctcccagcccgaacatgagttcgacagctccaagttctatgacgtaagaccttgtctcaggcggaatcggtgctgtactgactggctgtgaaggatatcatctataaaacctctccgaatgaccctgatgcccctgtgtatctacaaccggactccaaagcttcaacggctacaggggatgggatctccctcctcaataccctattgtctagtgtcaactcaagatccgtgcctcggcgcactcatttctcgaatatgccgctggagcttggacccaacctcaaaatctcagtgtcaggctatatcctctttcggcggcaagcgcccgcccggaactgctatgtctggcttggaggcgagaagcccgagattgtcaaaggagtcacgactcaaatagccgacgacacggcgcgcacggtggagaaatgggagatcagaaaggcctacaagttcggcggggaccaagttgtctttacccccgaggagcagaaggagttgaaaaacttcggtgatccggtcatccgcattataggcttcaagcccgcttctgccattccctactgggcgaacatgaaacatccttatttcatatatccgtcagaggaggactacgtgggttcaacccgcgtgttctccgccttgcatcagacgcttctgcggcagaagaagatagctctcgtctggttcattccacggagggctgccaacccggtccttggtgctatgatcgccggagaggagaaggtcgatgagaacggcgtgcagaagtacccccctggcatgtggattgtgccacttccgtacgccgatgatgttcgccagaaccccgagaccaccctgaatgtggctccagaaccgttgatcgaccagatgcgtgttattgtccagcagctgcaactccccaaggcctgctacgagcctctgaaatacccaaatccatgtaagtgtttgaattgccctttgatccgcgcgtcattggtcattgactaacttgttttagcattacaatggcactatcgcatcttacaggcgctggctctggacgaggatcttcctgagagaccggaagacaagaccgtcccgaagtacagacagattgacaaggtacgatacttcgcttttgatactatgactgtcactaattttcaatgccagcgcgctggggactatgtgctgtcatgggccgacgagctcgagaagcagtacgccacgatcgccgttgagaaaccagcatccagcactcttgtcaagcgaggcgcgaagaatcgtgccccggaagacgacgcagagtccagcaagccagctaagaaggtcaaagtggaagccgacaataacattgaggaggaagtgcggcgacattaccagaagaacaacctgtccagggtaactattatcttgccatgcggtgtgtgaccacgctaatatgttgtgcagcttacggtgaatatcctgaaggatttcctcacgtctcatggacgctctggggtggggaagaaggcagatctgatcgatcgcgtggagcaattcttggagtctggataa

SEQ ID NO: 5 - DNA, 897 bp, Aspergillus aculeatinus PF1378
  source 1..897: mol_type = genomic DNA
atgtcgtccaagtcgcaattgacctacactgcccgtgcgagcaagcacaacaaccctctggccaagcgcctcttcgagatcgccgaggccaagaagaccaatgtgaccgtctccgccgacgtgaccactaccaaggagctcctggacctcgctgaccgtaggcccgccgaaacctctttcactccatgataaggaattgacccccgagatatgtacataggcctgggaccctacatcgccgtgatcaagacgcacatcgacattctgtcggacttcagcaacgagaccatcgagggcctcaaggcgctgtccgagaagcacaacttcctgatcttcgaggaccgcaagttcatcgacatcggcaacaccgtccagaagcagtaccacaagggcaccctccggatctcggagtgggcccacatcatcaactgcagcatcctgcccggcgagggcatcgtggaggccctggcccagaccgccgctgccgaggacttcgagtacggcgccgagcgcggcctcctgatcctggccgagatgacctccaagggatccctcgccacgggccagtacaccaccgcctcggtggactacgcgcgcaaataccagaagttcgtcatggggttcgtgtccacgcgggcgctgggcgaggtgcagtcggaggcgagctccgcctcggaggaggaggactttgtcgtgttcacgacgggcgtcaatatctcctccaagggcgataagctcggccagcagtaccagacccccgcctctgcgattggtcgcggagccgatttcatcatcgccggtcgcgggatctatgccgcggcggacccggtgcaggcggcgcagcagtaccagaaggagggctgggaggcgtaccaggcccgtgttggcggaaactaa

SEQ ID NO: 6 - DNA, 810 bp, Aspergillus aculeatinus PF1378
  source 1..810: mol_type = other DNA
atgtcagacctgtacgagcagcgcatgccgcgctgcgaagctgaggccgagagcaacctcggctacgacctgcatcccagcgtcgagcaagagctccccgcagacgcacgcatcgccgacatagccaccggcacgggcatcttcctgcggcgaatcgcacccagcttcccggacgcggtcctccacggctacgacatttccgccactctatacccgcccaagtccgccctcgcgcccaacatcgacctccaagtcctcgacgccaagcagcagattcccctccacctgcaggggcagtacgatttggtccacgtccgcaatatctccatgggcctgatgccggacgaatggccggcgctggtggccaacctggtcacactgctcaagcccggcggcgtgctgcaatgggtggaatgcgacgcattgcacgtgcagcatctcggatccagccagggctcgaccaccgcggctctggagacgatgtatggcatgaatcgcgcgctggtcaaatcgcggttcgaggggggctggaccaccttgccggggatcctggagcgactgagactagtggatgtcgaacatcacaccgtgggcacggatcgggtggcctggacgcggtccaagctgaccgctaatagtatgacctttgcttttctgtctgcacgcgcggggaaggcgggagatgggcctgcgttgagtgggaaggagattgatcggttggaagagcaggtgaggatggatatcgagtccgggggctatttgcggtatgatattcattgctttctggctgttaagccgcatcttaactag

SEQ ID NO: 7 - protein, 269 aa, Aspergillus aculeatinus PF1378
MSDLYEQRMPRCEAEAESNLGYDLHPSVEQELPADARIADIATGTGIFLRRIAPSFPDAVLHGYDISATLYPPKSALAPNIDLQVLDAKQQIPLHLQGQYDLVHVRNISMGLMPDEWPALVANLVTLLKPGGVLQWVECDALHVQHLGSSQGSTTAALETMYGMNRALVKSRFEGGWTTLPGILERLRLVDVEHHTVGTDRVAWTRSKLTANSMTFAFLSARAGKAGDGPALSGKEIDRLEEQVRMDIESGGYLRYDIHCFLAVKPHLN

SEQ ID NO: 8 - DNA, 939 bp, Aspergillus aculeatinus PF1378
  source 1..939: mol_type = genomic DNA
atgtcagacctgtacgagcagcgcatgccgcgctgcgaagctgaggccgagaggttcgtgaaccaatcgaatctcgatcgccggacatcattaacgcgcgtctagactcgacgagcaatactccctgcatggagcgtgcgtagcccaactctcccctcccaaccggcgtctaacccatccagcaacctcggctacgacctgcatcccagcgtcgagcaagagctccccgcagacgcacgcatcgccgacatagccaccggcacgggcatcttcctgcggcgaatcgcacccagcttcccggacgcggtcctccacggctacgacatttccgccactctatacccgcccaagtccgccctcgcgcccaacatcgacctccaagtcctcgacgccaagcagcagattcccctccacctgcaggggcagtacgatttggtccacgtccgcaatatctccatgggcctgatgccggacgaatggccggcgctggtggccaacctggtcacactgctcaagcccggcggcgtgctgcaatgggtggaatgcgacgcattgcacgtgcagcatctcggatccagccagggctcgaccaccgcggctctggagacgatgtatggcatgaatcgcgcgctggtcaaatcgcggttcgaggggggctggaccaccttgccggggatcctggagcgactgagactagtggatgtcgaacatcacaccgtgggcacggatcgggtggcctggacgcggtccaagctgaccgctaatagtatgacctttgcttttctgtctgcacgcgcggggaaggcgggagatgggcctgcgttgagtgggaaggagattgatcggttggaagagcaggtgaggatggatatcgagtccgggggctatttgcggtatgatattcattgctttctggctgttaagccgcatcttaactag

SEQ ID NO: 9 - DNA, 1012 bp, Aspergillus aculeatinus PF1378
  source 1..1012: mol_type = genomic DNA
atttgttgctgctgctgctgctgctgctgctgcggcggcggcggcggcggcgaccgcgaggttgacctcacatcccaccgagcccacagtggatcggggcgggcgccactcggccgtgccacagctgcccttccaacagacaaatcaacgttgccacctgccgcggggttctgttgcaaacaaggccaacaaaagtcggaccagcagcaaaaatccactccttacctgcgttgatgcccagaatttcagtccaaaccgaggggtacttgcgggaaccttgaactgtagtacctacgtgctgcaacccccaccttgagtttacggatttggtagtatgtagccagctggaggcgatttttgagagagaggaaccaaagaagaggatagggggtaataccgactaccgagtatctggataggtggaaagaagggaaaatggtaggtaaagaaaagaaaaaaaaaaaattcttcgatatagtggatacggttgcaaataaggactccgagtggttcaaaatgaatagacaggataagcagaaccaagtaatgatcgcatgggctctgctcagtctactcagtctgctccatgctgcaagcagtccaggctccgcccagcaggtgaagatttttttttgcgctgggcccgcatttggaaccaaccagactggaagtggggctgggtcaacctggtttacccctccatgtccaattgcgctcattattcgccaagggttggagcccgcccgcttagtcgccctctcgcttgacccctccatataaggatttcccctcctccccctcccacagaattttcttccttccctcctcgtccgcttcagtacgtatatctttcccccctccttctcgcttccctcttccctcttcttcttcctttcttcattcctgtcttactgactcttgttgttcagcacctctacgcatttgtggccgtagtatctgagcaatttttttttagaaccttttcaaaagttcacttcacaacaccgtcacc